European Patent Application EP 4 729 545 A1, published April 22, 2026. Title: Anti-VEGF-anti-PD-L1 bispecific antibody, pharmaceutical composition of same and uses thereof. Applicant: BIOTHEUS INC. The sequence listing filed with the application follows.

SEQUENCE LISTING (31 sequences)

SEQ ID NO: 1 - protein, 578 aa, synthetic construct
EVQLVESGGGLVQPGGSLRLSCAASGYTFTNYGMNWVRQAPGKGLEWVGWINTYTGEPTYAADFKRRFTFSLDTSKSTAYLQMNSLRAEDTAVYYCAKYPHYYGSSHWYFDVWGQGTLVTVSSASTKGPSVFPLAPSSKSTSGGTAALGCLVKDYFPEPVTVSWNSGALTSGVHTFPAVLQSSGLYSLSSVVTVPSSSLGTQTYICNVNHKPSNTKVDKKVEPKSCDKTHTCPPCPAPEAAGGPSVFLFPPKPKDTLMISRTPEVTCVVVDVSHEDPEVKFNWYVDGVEVHNAKTKPREEQYNSTYRVVSVLTVLHQDWLNGKEYKCKVSNKALPAPIEKTISKAKGQPREPQVYTLPPSRDELTKNQVSLTCLVKGFYPSDIAVEWESNGQPENNYKTTPPVLDSDGSFFLYSKLTVDKSRWQQGNVFSCSVMHEALHNHYTQKSLSLSPGGGGGSGGGGSGEVQLQESGGGLVQPGGSLRLSCAASGFTFSSYWMYWLRQAPGKGLEWVSSINSDSSSTYYRDSVKGRFTISRDNAKNTLYLQMNSLKSEDTAVYYCAKDPGGYAKGQGTQVTVSS

SEQ ID NO: 2 - protein, 588 aa, synthetic construct
EVQLVESGGGLVQPGGSLRLSCAASGYTFTNYGMNWVRQAPGKGLEWVGWINTYTGEPTYAADFKRRFTFSLDTSKSTAYLQMNSLRAEDTAVYYCAKYPHYYGSSHWYFDVWGQGTLVTVSSASTKGPSVFPLAPSSKSTSGGTAALGCLVKDYFPEPVTVSWNSGALTSGVHTFPAVLQSSGLYSLSSVVTVPSSSLGTQTYICNVNHKPSNTKVDKKVEPKSCDKTHTCPPCPAPEAAGGPSVFLFPPKPKDTLMISRTPEVTCVVVDVSHEDPEVKFNWYVDGVEVHNAKTKPREEQYNSTYRVVSVLTVLHQDWLNGKEYKCKVSNKALPAPIEKTISKAKGQPREPQVYTLPPSRDELTKNQVSLTCLVKGFYPSDIAVEWESNGQPENNYKTTPPVLDSDGSFFLYSKLTVDKSRWQQGNVFSCSVMHEALHNHYTQKSLSLSPGGGGGSGGGGSGGGGSGGGGSGEVQLQESGGGLVQPGGSLRLSCAASGFTFSSYWMYWLRQAPGKGLEWVSSINSDSSSTYYRDSVKGRFTISRDNAKNTLYLQMNSLKSEDTAVYYCAKDPGGYAKGQGTQVTVSS

SEQ ID NO: 3 - protein, 123 aa, synthetic construct [sequence omitted]

SEQ ID NO: 4 - protein, 329 aa, synthetic construct
ASTKGPSVFPLAPSSKSTSGGTAALGCLVKDYFPEPVTVSWNSGALTSGVHTFPAVLQSSGLYSLSSVVTVPSSSLGTQTYICNVNHKPSNTKVDKKVEPKSCDKTHTCPPCPAPEAAGGPSVFLFPPKPKDTLMISRTPEVTCVVVDVSHEDPEVKFNWYVDGVEVHNAKTKPREEQYNSTYRVVSVLTVLHQDWLNGKEYKCKVSNKALPAPIEKTISKAKGQPREPQVYTLPPSRDELTKNQVSLTCLVKGFYPSDIAVEWESNGQPENNYKTTPPVLDSDGSFFLYSKLTVDKSRWQQGNVFSCSVMHEALHNHYTQKSLSLSPG

SEQ ID NO: 5 - protein, 115 aa, synthetic construct
EVQLQESGGGLVQPGGSLRLSCAASGFTFSSYWMYWLRQAPGKGLEWVSSINSDSSSTYYRDSVKGRFTISRDNAKNTLYLQMNSLKSEDTAVYYCAKDPGGYAKGQGTQVTVSS

SEQ ID NO: 6 - protein, 11 aa, synthetic construct
GGGGSGGGGSG

SEQ ID NO: 7 - protein, 21 aa, synthetic construct
GGGGSGGGGSGGGGSGGGGSG

SEQ ID NO: 8 - protein, 214 aa, synthetic construct
DIQMTQSPSSLSASVGDRVTITCSASQDISNYLNWYQQKPGKAPKVLIYFTSSLHSGVPSRFSGSGSGTDFTLTISSLQPEDFATYYCQQYSTVPWTFGQGTKVEIKRTVAAPSVFIFPPSDEQLKSGTASVVCLLNNFYPREAKVQWKVDNALQSGNSQESVTEQDSKDSTYSLSSTLTLSKADYEKHKVYACEVTHQGLSSPVTKSFNRGEC

SEQ ID NO: 9 - protein, 107 aa, synthetic construct [sequence omitted]

SEQ ID NO: 10 - protein, 107 aa, synthetic construct [sequence omitted]

SEQ ID NO: 11 - protein, 578 aa, synthetic construct
EVQLVESGGGLVQPGGSLRLSCAASGYDFTHYGMNWVRQAPGKGLEWVGWINTYTGEPTYAADFKRRFTFSLDTSKSTAYLQMNSLRAEDTAVYYCAKYPYYYGTSHWYFDVWGQGTLVTVSSASTKGPSVFPLAPSSKSTSGGTAALGCLVKDYFPEPVTVSWNSGALTSGVHTFPAVLQSSGLYSLSSVVTVPSSSLGTQTYICNVNHKPSNTKVDKKVEPKSCDKTHTCPPCPAPEAAGGPSVFLFPPKPKDTLMISRTPEVTCVVVDVSHEDPEVKFNWYVDGVEVHNAKTKPREEQYNSTYRVVSVLTVLHQDWLNGKEYKCKVSNKALPAPIEKTISKAKGQPREPQVYTLPPSRDELTKNQVSLTCLVKGFYPSDIAVEWESNGQPENNYKTTPPVLDSDGSFFLYSKLTVDKSRWQQGNVFSCSVMHEALHNHYTQKSLSLSPGGGGGSGGGGSGEVQLQESGGGLVQPGGSLRLSCAASGFTFSSYWMYWLRQAPGKGLEWVSSINSDSSSTYYRDSVKGRFTISRDNAKNTLYLQMNSLKSEDTAVYYCAKDPGGYAKGQGTQVTVSS

SEQ ID NO: 12 - protein, 588 aa, synthetic construct
EVQLVESGGGLVQPGGSLRLSCAASGYDFTHYGMNWVRQAPGKGLEWVGWINTYTGEPTYAADFKRRFTFSLDTSKSTAYLQMNSLRAEDTAVYYCAKYPYYYGTSHWYFDVWGQGTLVTVSSASTKGPSVFPLAPSSKSTSGGTAALGCLVKDYFPEPVTVSWNSGALTSGVHTFPAVLQSSGLYSLSSVVTVPSSSLGTQTYICNVNHKPSNTKVDKKVEPKSCDKTHTCPPCPAPEAAGGPSVFLFPPKPKDTLMISRTPEVTCVVVDVSHEDPEVKFNWYVDGVEVHNAKTKPREEQYNSTYRVVSVLTVLHQDWLNGKEYKCKVSNKALPAPIEKTISKAKGQPREPQVYTLPPSRDELTKNQVSLTCLVKGFYPSDIAVEWESNGQPENNYKTTPPVLDSDGSFFLYSKLTVDKSRWQQGNVFSCSVMHEALHNHYTQKSLSLSPGGGGGSGGGGSGGGGSGGGGSGEVQLQESGGGLVQPGGSLRLSCAASGFTFSSYWMYWLRQAPGKGLEWVSSINSDSSSTYYRDSVKGRFTISRDNAKNTLYLQMNSLKSEDTAVYYCAKDPGGYAKGQGTQVTVSS

SEQ ID NO: 13 - protein, 123 aa, synthetic construct [sequence omitted]

SEQ ID NO: 14 - protein, 214 aa, synthetic construct
DIQLTQSPSSLSASVGDRVTITCSASQDISNYLNWYQQKPGKAPKVLIYFTSSLHSGVPSRFSGSGSGTDFTLTISSLQPEDFATYYCQQYSTVPWTFGQGTKVEIKRTVAAPSVFIFPPSDEQLKSGTASVVCLLNNFYPREAKVQWKVDNALQSGNSQESVTEQDSKDSTYSLSSTLTLSKADYEKHKVYACEVTHQGLSSPVTKSFNRGEC

SEQ ID NO: 15 - protein, 107 aa, synthetic construct [sequence omitted]

SEQ ID NO: 16 - protein, 567 aa, synthetic construct
EVQLQESGGGLVQPGGSLRLSCAASGFTFSSYWMYWLRQAPGKGLEWVSSINSDSSSTYYRDSVKGRFTISRDNAKNTLYLQMNSLKSEDTAVYYCAKDPGGYAKGQGTQVTVSSDKTHTCPPCPAPEAAGGPSVFLFPPKPKDTLMISRTPEVTCVVVDVSHEDPEVKFNWYVDGVEVHNAKTKPREEQYNSTYRVVSVLTVLHQDWLNGKEYKCKVSNKALPAPIEKTISKAKGQPREPQVYTLPPSRDELTKNQVSLTCLVKGFYPSDIAVEWESNGQPENNYKTTPPVLDSDGSFFLYSKLTVDKSRWQQGNVFSCSVMHEALHNHYTQKSLSLSPGGGGGSGGGGSGGGGSGGGGSGSDTGRPFVEMYSEIPEIIHMTEGRELVIPCRVTSPNITVTLKKFPLDTLIPDGKRIIWDSRKGFIISNATYKEIGLLTCEATVNGHLYKTNYLTHRQTNTIIDVVLSPSHGIELSVGEKLVLNCTARTELNVGIDFNWEYPSSKHQHKKLVNRDLKTQSGSEMKKFLSTLTIDGVTRSDQGLYTCAASSGLMTKKNSTFVRVHEK

SEQ ID NO: 17 - protein, 205 aa, synthetic construct
SDTGRPFVEMYSEIPEIIHMTEGRELVIPCRVTSPNITVTLKKFPLDTLIPDGKRIIWDSRKGFIISNATYKEIGLLTCEATVNGHLYKTNYLTHRQTNTIIDVVLSPSHGIELSVGEKLVLNCTARTELNVGIDFNWEYPSSKHQHKKLVNRDLKTQSGSEMKKFLSTLTIDGVTRSDQGLYTCAASSGLMTKKNSTFVRVHEK

SEQ ID NO: 18 - protein, 226 aa, synthetic construct
DKTHTCPPCPAPEAAGGPSVFLFPPKPKDTLMISRTPEVTCVVVDVSHEDPEVKFNWYVDGVEVHNAKTKPREEQYNSTYRVVSVLTVLHQDWLNGKEYKCKVSNKALPAPIEKTISKAKGQPREPQVYTLPPSRDELTKNQVSLTCLVKGFYPSDIAVEWESNGQPENNYKTTPPVLDSDGSFFLYSKLTVDKSRWQQGNVFSCSVMHEALHNHYTQKSLSLSPG

SEQ ID NO: 19 - protein, 567 aa, synthetic construct
SDTGRPFVEMYSEIPEIIHMTEGRELVIPCRVTSPNITVTLKKFPLDTLIPDGKRIIWDSRKGFIISNATYKEIGLLTCEATVNGHLYKTNYLTHRQTNTIIDVVLSPSHGIELSVGEKLVLNCTARTELNVGIDFNWEYPSSKHQHKKLVNRDLKTQSGSEMKKFLSTLTIDGVTRSDQGLYTCAASSGLMTKKNSTFVRVHEKDKTHTCPPCPAPEAAGGPSVFLFPPKPKDTLMISRTPEVTCVVVDVSHEDPEVKFNWYVDGVEVHNAKTKPREEQYNSTYRVVSVLTVLHQDWLNGKEYKCKVSNKALPAPIEKTISKAKGQPREPQVYTLPPSRDELTKNQVSLTCLVKGFYPSDIAVEWESNGQPENNYKTTPPVLDSDGSFFLYSKLTVDKSRWQQGNVFSCSVMHEALHNHYTQKSLSLSPGGGGGSGGGGSGGGGSGGGGSGEVQLQESGGGLVQPGGSLRLSCAASGFTFSSYWMYWLRQAPGKGLEWVSSINSDSSSTYYRDSVKGRFTISRDNAKNTLYLQMNSLKSEDTAVYYCAKDPGGYAKGQGTQVTVSS

SEQ ID NO: 20 - protein, 108 aa, synthetic construct
ASTKGPSVFPLAPSSKSTSGGTAALGCLVKDYFPEPVTVSWNSGALTSGVHTFPAVLQSSGLYSLSSVVTVPSSSLGTQTYICNVNHKPSNTKVDKKVEPKSCDKTHT

SEQ ID NO: 21 - protein, 8 aa, synthetic construct
GYTFTNYG

SEQ ID NO: 22 - protein, 9 aa, synthetic construct
INTYTGEPT

SEQ ID NO: 23 - protein, 16 aa, synthetic construct
AKYPHYYGSSHWYFDV

SEQ ID NO: 24 - protein, 6 aa, synthetic construct
QDISNY

SEQ ID NO: 25 - skipped

SEQ ID NO: 26 - protein, 9 aa, synthetic construct
QQYSTVPWT

SEQ ID NO: 27 - protein, 8 aa, synthetic construct
GYDFTHYG

SEQ ID NO: 28 - protein, 16 aa, synthetic construct
AKYPYYYGTSHWYFDV

SEQ ID NO: 29 - protein, 8 aa, synthetic construct
GFTFSSYW

SEQ ID NO: 30 - protein, 8 aa, synthetic construct
INSDSSST

SEQ ID NO: 31 - protein, 8 aa, synthetic construct
AKDPGGYA